European Patent Application EP 4 650 446 A1, published November 19, 2025. Title: 一种用于抑制细胞程序性死亡-配体1基因表达的siRNA、其缀合物和药物组合物及用途. Applicant: 苏州时安生物技术有限公司. Application CN. The sequence listing filed with the application follows.

SEQUENCE LISTING (28 sequences)

SEQ ID NO: 1 - RNA, 19 nt, synthetic construct
  source 1..19: mol_type = other RNA
tatttgctgtctttatatt

SEQ ID NO: 2 - RNA, 19 nt, synthetic construct
  source 1..19: mol_type = other RNA
tttgctgtctttatattca

SEQ ID NO: 3 - RNA, 19 nt, synthetic construct
  source 1..19: mol_type = other RNA
agatgaggatatttgctgt

SEQ ID NO: 4 - RNA, 19 nt, synthetic construct
  source 1..19: mol_type = other RNA
aagatgaggatatttgcta

SEQ ID NO: 5 - RNA, 19 nt, synthetic construct
  source 1..19: mol_type = other RNA
atgaggatatttgctgtct

SEQ ID NO: 6 - RNA, 19 nt, synthetic construct
  source 1..19: mol_type = other RNA
gatatttgctgtctttata

SEQ ID NO: 7 - RNA, 19 nt, synthetic construct
  source 1..19: mol_type = other RNA
ccagaaagatgaggatatt

SEQ ID NO: 8 - RNA, 19 nt, synthetic construct
  source 1..19: mol_type = other RNA
gaggatatttgctgtcttt

SEQ ID NO: 9 - RNA, 19 nt, synthetic construct
  source 1..19: mol_type = other RNA
ctcaatgcctcaatttgtt

SEQ ID NO: 10 - RNA, 19 nt, synthetic construct
  source 1..19: mol_type = other RNA
tatttgctgtctttatata

SEQ ID NO: 11 - RNA, 19 nt, synthetic construct
  source 1..19: mol_type = other RNA
agatgaggatatttgctga

SEQ ID NO: 12 - RNA, 19 nt, synthetic construct
  source 1..19: mol_type = other RNA
gaggatatttgctgtctta

SEQ ID NO: 13 - RNA, 21 nt, synthetic construct
  source 1..21: mol_type = other RNA
aatataaagacagcaaatatc

SEQ ID NO: 14 - RNA, 21 nt, synthetic construct
  source 1..21: mol_type = other RNA
tgaatataaagacagcaaata

SEQ ID NO: 15 - RNA, 21 nt, synthetic construct
  source 1..21: mol_type = other RNA
acagcaaatatcctcatcttt

SEQ ID NO: 16 - RNA, 21 nt, synthetic construct
  source 1..21: mol_type = other RNA
tagcaaatatcctcatctttc

SEQ ID NO: 17 - RNA, 21 nt, synthetic construct
  source 1..21: mol_type = other RNA
agacagcaaatatcctcatct

SEQ ID NO: 18 - RNA, 21 nt, synthetic construct
  source 1..21: mol_type = other RNA
tataaagacagcaaatatcct

SEQ ID NO: 19 - RNA, 21 nt, synthetic construct
  source 1..21: mol_type = other RNA
aatatcctcatctttctggaa

SEQ ID NO: 20 - RNA, 21 nt, synthetic construct
  source 1..21: mol_type = other RNA
aaagacagcaaatatcctcat

SEQ ID NO: 21 - RNA, 21 nt, synthetic construct
  source 1..21: mol_type = other RNA
aacaaattgaggcattgagtg

SEQ ID NO: 22 - RNA, 21 nt, synthetic construct
  source 1..21: mol_type = other RNA
tatataaagacagcaaatatc

SEQ ID NO: 23 - RNA, 21 nt, synthetic construct
  source 1..21: mol_type = other RNA
tcagcaaatatcctcatcttt

SEQ ID NO: 24 - RNA, 21 nt, synthetic construct
  source 1..21: mol_type = other RNA
taagacagcaaatatcctcat

SEQ ID NO: 25 - RNA, 19 nt, synthetic construct
  source 1..19: mol_type = other RNA
gttttctgctttctgtcaa

SEQ ID NO: 26 - RNA, 21 nt, synthetic construct
  source 1..21: mol_type = other RNA
ttgacagaaagcagaaaacaa

SEQ ID NO: 27 - RNA, 19 nt, synthetic construct
  source 1..19: mol_type = other RNA
gagattagatcctgaggaa

SEQ ID NO: 28 - RNA, 21 nt, synthetic construct
  source 1..21: mol_type = other RNA
ttcctcaggatctaatctcct